European Patent Specification EP 3 554 470 B1, published July 26, 2023. Title: Cosmetic Compositions. Applicant: Shah, Snehal Wang, Hua Xu, Zhequan Smail, Mary Ann Sojka, Milan Franz Bratescu, Daniela. The sequence listing filed with the application follows.

SEQUENCE LISTING (7 sequences)

SEQ ID NO: 1 - protein, 13 aa, Artificial Sequence
  CLOCK and/or PER1 gene activator
  misc_feature (1)..(4): Xaa can be any naturally occurring amino acid or no amino acid 220>
  misc_feature (5): Xaa can be threonine or serine or no amino acid
  misc_feature (9): Xaa can be isoleucine, leucine, proline, valine, alanine, glycine or no amino acid
  misc_feature (10)..(13): Xaa can be any naturally occurring amino acid or no amino acid
XXXXXSTPXXXXX

SEQ ID NO: 2 - protein, 7 aa, Artificial Sequence
  CLOCK and/or PER1 gene activator
YVSTPYN

SEQ ID NO: 3 - protein, 5 aa, Artificial Sequence
  CLOCK and/or PER1 gene activator
VSTPE

SEQ ID NO: 4 - protein, 6 aa, Artificial Sequence
  CLOCK and/or PER1 gene activator
LHSTPP

SEQ ID NO: 5 - protein, 6 aa, Artificial Sequence
  CLOCK and/or PER1 gene activator
RHSTPE

SEQ ID NO: 6 - protein, 5 aa, Artificial Sequence
  CLOCK and/or PER1 gene activator
HSTPE

SEQ ID NO: 7 - protein, 4 aa, Artificial Sequence
  CLOCK and/or PER1 gene activator
SPLQ